European Patent Specification EP 3 409 116 B1, published August 9, 2023. Title: An agent for improving heat stress resistance in plants, a method for improving heat stress resistance in plants, an agent for suppressing whitening of plants, and an agent for enhancing expression of DREB2A gene in plants. Applicant: Kaneka Corporation. The sequence listing filed with the application follows.

SEQUENCE LISTING (2 sequences)

SEQ ID NO: 1 - DNA, 1450 bp, Arabidopsis thaliana (ecotype: Columbia)
agatattttgatttctgctaaagctgtctgataaaaagaagaggaaaactcgaaaaagctacacacaagaagaagaagaaaagatacgagcaagaagactaaacacgaaagcgatttatcaactcgaaggaagagactttgattttcaaatttcgtcccctatagattgtgttgtttctgggaaggagatggcagtttatgatcagagtggagatagaaacagaacacaaattgatacatcgaggaaaaggaaatctagaagtagaggtgacggtactactgtggctgagagattaaagagatggaaagagtataacgagaccgtagaagaagtttctaccaagaagaggaaagtacctgcgaaagggtcgaagaagggttgtatgaaaggtaaaggaggaccagagaatagccgatgtagtttcagaggagttaggcaaaggatttggggtaaatgggttgctgagatcagagagcctaatcgaggtagcaggctttggcttggtactttccctactgctcaagaagctgcttctgcttatgatgaggctgctaaagctatgtatggtcctttggctcgtcttaatttccctcggtctgatgcgtctgaggttacgagtacctcaagtcagtctgaggtgtgtactgttgagactcctggttgtgttcatgtgaaaacagaggatccagattgtgaatctaaacccttctccggtggagtggagccgatgtattgtctggagaatggtgcggaagagatgaagagaggtgttaaagcggataagcattggctgagcgagtttgaacataactattggagtgatattctgaaagagaaagagaaacagaaggagcaagggattgtagaaacctgtcagcaacaacagcaggattcgctatctgttgcagactatggttggcccaatgatgtggatcagagtcacttggattcttcagacatgtttgatgtcgatgagcttctacgtgacctaaatggcgacgatgtgtttgcaggcttaaatcaggaccggtacccggggaacagtgttgccaacggttcatacaggcccgagagtcaacaaagtggttttgatccgctacaaagcctcaactacggaatacctccgtttcagctcgagggaaaggatggtaatggattcttcgacgacttgagttacttggatctggagaactaaacaaaacaatatgaagctttttggatttgatatttgccttaatcccacaacgactgttgattctctatccgagttttagtgatatagagaactacagaacacgttttttcttgttataaaggtgaactgtatatatcgaaacagtgatatgacaatagagaagacaactatagtttgttagtctgcttctcttaagttgttctttagatatgttttatgttttgtaacaacaggaatgaataatacacacttgt

SEQ ID NO: 2 - DNA, 1833 bp, Arabidopsis thaliana (ecotype: Columbia)
atgcctgcttttcttcagctttaagggaaaagatcaaagattgggtcttcaacacttgagagagtctctgtctctgtaaaagatatttgagcttgagaagaacagaagaaacttccaggatcaatcaatcgatcaactttagtgaactaactcttgatttttcattcgaagttatggaatcggttcccgaatccgtaccatcgccgaactcgaatacaccgtcaataccaccgccggtgaactccgtaccgcctttcttgagtaaaacctacgacatggttgatgatccgttgaccaatgaggtcgtttcgtggagcagcgggaacaacagcttcgtcgtctggagtgccccggagttctcgaaggtgctcttgcccaagtatttcaagcacaacaacttctccagcttcgtcagacagttaaatacttatggtttcagaaaagttgatcctgaccgatgggaatttgcaaatgaaggatttcttagaggccgaaaacaactactgaagagtattgtcaggagaaaaccttcgcatgtgcagcagaatcagcaacaaactcaagttcagagctcatctgttggtgcttgtgtcgaggtggggaagtttggaatagaagaagaagtggaaagacttaagcgggataagaatgttcttatgcaagaactcgtcaggttaaggcagcaacagcaagctactgaaaaccaactgcagaatgtgggacagaaagttcaggtgatggagcaaaggcaacaacaaatgatgtcgtttttagcaaaggctgttcaaagtccaggtttcttaaaccagttagtacaacagaataataatgatggcaacagacaaattccaggaagcaacaaaaagaggagacttcctgtagatgagcaggagaatcgtggtgacaatgtggctaatggtcttaaccgccagattgttagatatcagccgtcgataaacgaagcagcacaaaatatgcttcgacagttcttaaatactagtacctcacctcggtatgaatcagtttcaaacaatcctgacagtttcctattgggtgatgttcccagttctacctctgtagacaatgggaacccttcaagtagagtttctggagtaacattggccgagttttcacccaacacagttcagtcagcaacgaatcaagtacccgaagcaagtttggctcatcatcctcaagctggtctggttcagccaaatataggtcaaagtccggctcaaggagcagcacctgcagactcttggagccctgaatttgatttagttggatgcgagacagatagtggagagtgttttgatccaataatggctgttttagatgagtcagaaggcgatgcaatttctcctgaaggtgagggcaagatgaatgagttactggagggagtccctaagctgcccggaatccaagatccattctgggaacagttcttttctgttgaactcccagcgattgcagatacagacgatattctatcaggatcagtggagaataatgacttggtattggaacaagaaccaaacgagtggacccgtaatgaacaacaaatgaagtatcttactgaacaaatgggactgctttcctcagaagcacagaggaaataaagattttcaggggaggttgcaaaaggagatatgaaggaacgaggaatatatcagatggtgtgtataccctttacatttttacttaaatgaaaaaaaaacagagagaagaaacataaaagatttaccaccaagcttgtgaatagttagtagagatcggtttttgtgttgtttatattatacttttgtgtgaaaacgttcatcttgttcaattatc